European Patent Application EP 4 722 375 A1, published April 8, 2026. Title: Efficient in vitro transcription of artificial mRNA with highly modified 5' ends. Applicant: ExploRNA THERAPEUTICS SP. Z O. O. Application EP. The sequence listing filed with the application follows.

SEQUENCE LISTING (19 sequences)

SEQ ID NO: 1 - DNA, 17 bp, Escherichia virus T7
  source 1..17: mol_type = other DNA
taatacgactcactata

SEQ ID NO: 2 - DNA, 17 bp, Escherichia virus T7
  source 1..17: mol_type = genomic DNA
taatacgactcactatt

SEQ ID NO: 3 - DNA, 18 bp, synthetic construct
  source 1..18: mol_type = other DNA
taatacgactcactatat

SEQ ID NO: 4 - DNA, 20 bp, synthetic construct
  source 1..20: mol_type = other DNA
taatacgactcactataagg

SEQ ID NO: 5 - DNA, 20 bp, synthetic construct
  source 1..20: mol_type = other DNA
ccttatagtgagtcgtatta

SEQ ID NO: 6 - DNA, 20 bp, synthetic construct
  source 1..20: mol_type = other DNA
taatacgactcactattagg

SEQ ID NO: 7 - DNA, 20 bp, synthetic construct
  source 1..20: mol_type = other DNA
cctaatagtgagtcgtatta

SEQ ID NO: 8 - DNA, 20 bp, synthetic construct
  source 1..20: mol_type = other DNA
taatacgactcactataggg

SEQ ID NO: 9 - DNA, 20 bp, synthetic construct
  source 1..20: mol_type = other DNA
ccctatagtgagtcgtatta

SEQ ID NO: 10 - DNA, 20 bp, synthetic construct
  source 1..20: mol_type = other DNA
taatacgactcactataatg

SEQ ID NO: 11 - DNA, 20 bp, synthetic construct
  source 1..20: mol_type = other DNA
cattatagtgagtcgtatta

SEQ ID NO: 12 - DNA, 20 bp, synthetic construct
  source 1..20: mol_type = other DNA
taatacgactcactatatgg

SEQ ID NO: 13 - DNA, 20 bp, synthetic construct
  source 1..20: mol_type = other DNA
ccatatagtgagtcgtatta

SEQ ID NO: 14 - DNA, 20 bp, synthetic construct
  source 1..20: mol_type = other DNA
taatacgactcactataaga

SEQ ID NO: 15 - DNA, 20 bp, synthetic construct
  source 1..20: mol_type = other DNA
tcttatagtgagtcgtatta

SEQ ID NO: 16 - DNA, 20 bp, synthetic construct
  source 1..20: mol_type = other DNA
taatacgactcactatagag

SEQ ID NO: 17 - DNA, 20 bp, synthetic construct
  source 1..20: mol_type = other DNA
ctctatagtgagtcgtatta

SEQ ID NO: 18 - DNA, 20 bp, synthetic construct
  source 1..20: mol_type = other DNA
taatacgactcactataaag

SEQ ID NO: 19 - DNA, 20 bp, synthetic construct
  source 1..20: mol_type = other DNA
ctttatagtgagtcgtatta